European Patent Specification EP 3 681 911 B1, published November 27, 2024. Title: Binding proteins to the human thrombin receptor PAR4. Applicant: Monash University. Application AU2017903685. The sequence listing filed with the application follows.

SEQUENCE LISTING (109 sequences)

SEQ ID NO: 1 - protein, 6 aa, Homo sapiens
PRGYPG

SEQ ID NO: 2 - protein, 20 aa, Homo sapiens
GDDSTPSILPAPRGYPGQVC

SEQ ID NO: 3 - protein, 20 aa, Mus musculus
LKEPKSSDKPNPRGYPGKFC

SEQ ID NO: 4 - protein, 21 aa, Artificial Sequence
  sequence of hPAR4 (KLH) used as immunogen
  MISC_FEATURE (21)..(21): keyhole limpet hemocyanin (KLH)
GDDSTPSILPAPRGYPGQVCX

SEQ ID NO: 5 - protein, 21 aa, Artificial Sequence
  sequence of mPAR4 (KLH) used as an immunogen
  MISC_FEATURE (21)..(21): keyhole limpet hemocyanin (KLH)
LKEPKSSDKPNPRGYPGKFCX

SEQ ID NO: 6 - protein, 25 aa, Artificial Sequence
  sequence of mPAR4 biotin conjugate
  MISC_FEATURE (25)..(25): streptavidin-k/biotin
LKEPKSSDKPNPRGYPGKFCGGGGX

SEQ ID NO: 7 - protein, 25 aa, Artificial Sequence
  sequence of hPAR4 biotin conjugate
  MISC_FEATURE (25)..(25): streptavidin-k/biotin (SKB)
GDDSTPSILPAPRGYPGQVCGGGGX

SEQ ID NO: 8 - protein, 23 aa, Artificial Sequence
  sequence of hPAR3 biotin conjugate
  MISC_FEATURE (23)..(23): streptavidin-k/biotin (SKB)
AKPTLPIKTFRGAPPNSFGGGGX

SEQ ID NO: 9 - protein, 23 aa, Artificial Sequence
  sequence of hPAR2 biotin conjugate
  MISC_FEATURE (23)..(34): streptavidin-k/biotin (SKB)
  MISC_FEATURE (23)..(23): streptavidin-k/biotin (SKB)
SCSGTIQGTNRSSKGRSLGGGGX

SEQ ID NO: 10 - protein, 23 aa, Artificial Sequence
  sequence of hPAR1 biotin conjugate
  MISC_FEATURE (23)..(23): streptavidin-k/biotin (SKB)
SKATNATLDPRSFLLRNPGGGGX

SEQ ID NO: 11 - protein, 121 aa, Artificial Sequence
  VH of 5A.RC3
QVQLVESGGGVVQPGRSLRLSCAASGFTLSNYGMHWVRQAPGKGLEWVSVIWYDGSNKHYADSVKGRFTISRDNSKNTLYLQMNSLRAEDTAVYYCARESIVEVLPPFDYWGQGTLVTVSS

SEQ ID NO: 12 - protein, 107 aa, Artificial Sequence
  VL of 5A.RC3
KIVLTQSPGTLSLSPGERVTLSCRASQRVRNNYLAWFQQKPGQAPRLFIYGASSRATGIPDRFSGSGSGTDFIFTISRLEPEDFAVYYCQQYGNSYTFGQGTKLEIK

SEQ ID NO: 13 - protein, 8 aa, Artificial Sequence
  VH CRD1 of 5A.RC3
GFTLSNYG

SEQ ID NO: 14 - protein, 8 aa, Artificial Sequence
  VH CRD2 of 5A.RC3, 5G.RA1, 5G.RF6,
IWYDGSNK

SEQ ID NO: 15 - protein, 14 aa, Artificial Sequence
  VH CDR3 of 5A.RC3
ARESIVEVLPPFDY

SEQ ID NO: 16 - protein, 7 aa, Artificial Sequence
  VL CDR1 of 5A.RC3
QRVRNNY

SEQ ID NO: 17 - protein, 3 aa, Artificial Sequence
  VL CDR2 of 5A.RC3
GAS

SEQ ID NO: 18 - protein, 8 aa, Artificial Sequence
  VL CDR3 of 5A.RC3
QQYGNSYT

SEQ ID NO: 19 - protein, 385 aa, Homo sapiens
MWGRLLLWPLVLGFSLSGGTQTPSVYDESGSTGGGDDSTPSILPAPRGYPGQVCANDSDTLELPDSSRALLLGWVPTRLVPALYGLVLVVGLPANGLALWVLATQAPRLPSTMLLMNLAAADLLLALALPPRIAYHLRGQRWPFGEAACRLATAALYGHMYGSVLLLAAVSLDRYLALVHPLRARALRGRRLALGLCMAAWLMAAALALPLTLQRQTFRLARSDRVLCHDALPLDAQASHWQPAFTCLALLGCFLPLLAMLLCYGATLHTLAASGRRYGHALRLTAVVLASAVAFFVPSNLLLLLHYSDPSPSAWGNLYGAYVPSLALSTLNSCVDPFIYYYVSAEFRDKVRAGLFQRSPGDTVASKASAEGGSRGMGTHSSLLQ

SEQ ID NO: 20 - DNA, 363 bp, Artificial Sequence
  VH of 5A.RC3
caggtgcagttggtggagtcggggggaggcgtggtccagcctgggaggtccctgagactctcctgtgcagcgtctggattcaccctcagtaactatggcatgcactgggtccgccaggctccaggcaaggggctggaatgggtgtcagttatctggtatgatggaagtaataaacactatgcagactccgtgaagggccgattcaccatctccagagacaattccaagaacacgctttatctgcaaatgaacagcctgagagccgaggacacggctgtatattattgtgcgagagagagtattgtggaggtgcttcctccttttgactattggggccagggaaccctggtcaccgtctcctca

SEQ ID NO: 21 - DNA, 348 bp, Artificial Sequence
  VL of 5A.RC3
aaaattgtgttgacgcagtctccaggcaccctgtctttgtctccaggggaaagagtcaccctctcctgcagggccagtcagcgtgttaggaacaactacttagcctggttccaacagaaacctggccaggctcccaggcttttcatctatggtgcatccagcagggccactggcatcccagacaggttcagtggcagtgggtctgggacagacttcattttcaccatcagcagactggagcctgaagattttgcagtgtattactgtcagcagtatggtaactcgtacacttttggccaggggaccaagctggagatcaaacgggctgatgctgcaccaactgtatcc

SEQ ID NO: 22 - protein, 126 aa, Artificial Sequence
  VH of 5F.RF3
QVQLVQSGAEVKKPGASVKVSCKTSAYTFTNYGISWVRQAPGQGLEWMGWISPYNGNTNYAQKLQGRVTMTTDTSTRTAYMELRSLRSDDTAVYYCAREYNRSSRGRYYYYGMDVWGQGTTVTVSS

SEQ ID NO: 23 - protein, 108 aa, Artificial Sequence
  VL of 5F.RF3
EIVLTQSPGTLSLSPGERATLSCRASQSVSSNYLAWYQKKPGQAPRLLISGASSRATGIPDRFSGSGSGTDFTLTISRLEPEDFAVYYCQQYGSSPWTFGQGTKVEIK

SEQ ID NO: 24 - protein, 8 aa, Artificial Sequence
  VH CDR1 of 5F.RF3
AYTFTNYG

SEQ ID NO: 25 - protein, 8 aa, Artificial Sequence
  VH CDR2 of 5F.RF3
ISPYNGNT

SEQ ID NO: 26 - protein, 19 aa, Artificial Sequence
  VH CDR3 of 5F.RF3
AREYNRSSRGRYYYYGMDV

SEQ ID NO: 27 - protein, 7 aa, Artificial Sequence
  VL CDR1 of 5F.RF3
QSVSSNY

SEQ ID NO: 28 - protein, 3 aa, Artificial Sequence
  VL CDR2 of 5F.RF3, 5G.RA1, 5D.RH4, 5G.RF6, 5G.RD6, 5H.RA3, 5G.RG1, 5H.RG4
GAS

SEQ ID NO: 29 - protein, 9 aa, Artificial Sequence
  VL CDR3 of 5F.RF3
QQYGSSPWT

SEQ ID NO: 30 - DNA, 378 bp, Artificial Sequence
  VH of 5F.RF3
caggttcagctggtgcagtctggagctgaggtgaagaagcctggggcctcagtgaaggtctcctgcaagacttctgcttacacctttaccaactatggtatcagctgggtgcgacaggcccctggacaagggcttgagtggatgggatggatcagcccttacaacggcaacacaaactatgcacagaagctccagggcagagtcaccatgaccacagacacatccacgaggacagcgtacatggagctgaggagcctgagatctgacgacacggccgtatattactgtgcgagagagtataacaggtcgtcgaggggccgctactactactacggtatggacgtctggggccaagggaccacggtcaccgtctcctca

SEQ ID NO: 31 - DNA, 351 bp, Artificial Sequence
  VL of 5F.RF3
gaaattgtgttgacgcagtctccaggcaccctgtctttgtctccaggggaaagagccaccctctcctgcagggccagtcagagtgttagtagcaactacttagcctggtaccagaagaaacctggccaggctcccaggctcctcatctctggtgcatccagcagggccactggcatcccagacaggttcagcggcagtgggtctgggacagacttcactctcaccatcagtagactggagcctgaagattttgcagtgtattactgtcagcagtatggtagctcaccgtggacgttcggccaagggaccaaggtggaaatcaaacgggctgatgctgcaccaactgtatcc

SEQ ID NO: 32 - protein, 121 aa, Artificial Sequence
  VH of 5H.RD2
EVQLVESGGDLVKPGGSLRLSCSASGFTFFNTWMNWVRQAPGKGLEWVGRVKSKNDGGTKDYAAPVTGRFTISRDDSKDTLYLQMNSLKTEDTAVYYCTTDPHYDFWSAYWGQGTLVTVSS

SEQ ID NO: 33 - protein, 112 aa, Artificial Sequence
  VL of 5H.RD2
DIVMTQTPLSSPVTLGQPASISCRSSQSLVHSDGNTYLSWLQQRPGQPPRLLIYKISNRFSGVPDRFSGSGAGTDFTLKISRVEAEDVGFYYCLQATQFMYTFGQGTKLEIK

SEQ ID NO: 34 - protein, 8 aa, Artificial Sequence
  VH CDR1 of 5H.RD2
GFTFFNTW

SEQ ID NO: 35 - protein, 10 aa, Artificial Sequence
  VH CDR2 of 5H.RD2
VKSKNDGGTK

SEQ ID NO: 36 - protein, 12 aa, Artificial Sequence
  VH CDR3 of 5H.RD2
TTDPHYDFWSAY

SEQ ID NO: 37 - protein, 10 aa, Artificial Sequence
  VL CDR1 of 5H.RD2
QSLVHSDGNT

SEQ ID NO: 38 - protein, 3 aa, Artificial Sequence
  VL CDR2 of 5H.RD2
KIS

SEQ ID NO: 39 - protein, 9 aa, Artificial Sequence
  VL CDR3 of 5H.RD2
LQATQFMYT

SEQ ID NO: 40 - DNA, 363 bp, Artificial Sequence
  VH of 5H.RD2
gaggtgcagctggtggagtctgggggagacttggtcaagcctggggggtcccttagactctcctgttcagcctctggattcactttctttaacacctggatgaactgggtccgccaggctccagggaaggggctggagtgggttggccgtgttaaaagcaaaaatgatggtgggacaaaagactacgctgcacccgtgacaggcagattcaccatctcaagagatgattcaaaagacacgctgtatctgcaaatgaacagcctgaaaaccgaggacacagccgtgtattactgtaccacagatccccactacgatttttggagtgcctactggggccagggaaccctggtcaccgtctcctca

SEQ ID NO: 41 - DNA, 363 bp, Artificial Sequence
  VL of 5H.RD2
gatattgtgatgacccagactccactctcctcacctgtcacccttggacagccggcctccatctcctgcaggtctagtcaaagcctcgttcacagtgatggaaatacctacttgagttggcttcagcagaggccaggccagcctccaagactcctaatttataagatttctaaccggttctctggggtcccagacagattcagtggcagtggggcagggacagatttcacactgaaaatcagcagggtggaggctgaggatgtcgggttttattactgcctgcaagctacacaattcatgtacacttttggccaggggaccaagctggagatcaaacgggctgatgctgcaccaactgtatcc

SEQ ID NO: 42 - protein, 5 aa, Artificial Sequence
  epitope PAR4 sequence
APRGY

SEQ ID NO: 43 - protein, 8 aa, Artificial Sequence
  epitope PAR4 sequence
ILPAPRGY

SEQ ID NO: 44 - protein, 9 aa, Artificial Sequence
  epitope PAR4 sequence
APRGYPGQV

SEQ ID NO: 45 - protein, 122 aa, Artificial Sequence
  VH of 5I.RG1
QVQLQQWGAGLLKPSETLSLACAISSGSFSTYFWRWIRQPPGKGLEWIGEIIHTGSTTYNPSLKSRVTISVDTSKNQLSLKLSSVTAADTAVYYCAFEYSSSGGYYYGMDVWGQGTTVTVSS

SEQ ID NO: 46 - protein, 107 aa, Artificial Sequence
  VL of 5I.RG1
DIQMTQSPSSLSASVGDRVTITCRASQSISSYLNWYQQIPGKAPNLLIYAASSLRSGVPSRFSGSGSGTDFTLTISSLQPEDFATYYCQQTYSTPLTFGGGTKVEIK

SEQ ID NO: 47 - protein, 8 aa, Artificial Sequence
  VH CDR1 of 5I.RG1
SGSFSTYF

SEQ ID NO: 48 - protein, 7 aa, Artificial Sequence
  VH CDR2 of 5I.RG1
IIHTGST

SEQ ID NO: 49 - protein, 16 aa, Artificial Sequence
  VH CDR3 of 5I.RG1
AFEYSSSGGYYYGMDV

SEQ ID NO: 50 - protein, 6 aa, Artificial Sequence
  VL CDR1 of 5I.RG1
QSISSY

SEQ ID NO: 51 - protein, 3 aa, Artificial Sequence
  VL CDR2 of 5I.RG1, 5H.RH4, 5G.RC5, 5F.RE6, 5H.RF2
AAS

SEQ ID NO: 52 - protein, 9 aa, Artificial Sequence
  VL CDR3 of 5I.RG1
QQTYSTPLT

SEQ ID NO: 53 - protein, 121 aa, Artificial Sequence
  VH of 5G.RA1
QVQLVESGGGVVQPGRSLRLSCAASGFTFSSYGMHWVRQAPGKGLEWVAVIWYDGSNKYYADSVKGRFTISRDNSKNTLYLQMNSLRAEDTAVYYCARETALVRGVPFDYWGQGTLVTVSS

SEQ ID NO: 54 - protein, 107 aa, Artificial Sequence
  VL of 5G.RA1
EIVLTQSPGTLSLSPGERATLSCRTSQSVRSSYLAWYQQKPGQAPRLLIYGASSRATGIPDRFSGSGSGTDFTLTISRLEPEDFAVYYCQQYGSSYTFGQGTKLEIK

SEQ ID NO: 55 - protein, 8 aa, Artificial Sequence
  VH CDR1 of 5G.RA1, 5H.RA3, 5F.RE6
GFTFSSYG

SEQ ID NO: 56 - protein, 14 aa, Artificial Sequence
  VH CDR3 of 5G.RA1
ARETALVRGVPFDY

SEQ ID NO: 57 - protein, 7 aa, Artificial Sequence
  VL CDR1 of 5G.RA1, 5D.RH4, 5G.RF6, 5G.RD6, 5H.RA3, 5H.RG4, 5G.RC5
QSVRSSY

SEQ ID NO: 58 - protein, 8 aa, Artificial Sequence
  VL CDR3 of 5G.RA1, 5G.RF6, 5G.RD6, 5H.RA3, 5H.RG4, 5G.RC5
QQYGSSYT

SEQ ID NO: 59 - protein, 8 aa, Artificial Sequence
  VH CDR1 of 5D.RH4
GFTFSSDG

SEQ ID NO: 60 - protein, 8 aa, Artificial Sequence
  VH CDR2 of 5D.RH4
IWFDGRNK

SEQ ID NO: 61 - protein, 14 aa, Artificial Sequence
  VH CDR3 of 5D.RH4
ARESSISTRPPFDY

SEQ ID NO: 62 - protein, 8 aa, Artificial Sequence
  VL CDR3 of 5D.RH4, 5G.RG1
QQYGRSYT

SEQ ID NO: 63 - protein, 8 aa, Artificial Sequence
  VH CDR1 of 5H.RH4
GGSFSNYY

SEQ ID NO: 64 - protein, 7 aa, Artificial Sequence
  VH CDR2 of 5H.RH4
INHSGST

SEQ ID NO: 65 - protein, 17 aa, Artificial Sequence
  VH CDR3 of 5H.RH4
KVEHSSSSGHYYYGMDV

SEQ ID NO: 66 - protein, 6 aa, Artificial Sequence
  VL CDR1 of 5H.RH4
QTISYY

SEQ ID NO: 67 - protein, 9 aa, Artificial Sequence
  VL CDR3 of 5H.RH4
QQSYSTPLT

SEQ ID NO: 68 - protein, 8 aa, Artificial Sequence
  VH CDR1 of 5G.RF6
GFTFSNYG

SEQ ID NO: 69 - protein, 13 aa, Artificial Sequence
  VH CDR3 of 5G.RF6
ARETIMVRGVPFD

SEQ ID NO: 70 - protein, 8 aa, Artificial Sequence
  VH CDR1 of 5G.RD6
GFAFSSYG

SEQ ID NO: 71 - protein, 8 aa, Artificial Sequence
  VH CDR2 of 5G.RD6
IWYDGSNR

SEQ ID NO: 72 - protein, 14 aa, Artificial Sequence
  VH CDR3 of 5G.RD6
ARETAMVRGVPFDY

SEQ ID NO: 73 - protein, 8 aa, Artificial Sequence
  VH CDR2 of 5H.RA3, 5F.RE6
IWYDGTKK

SEQ ID NO: 74 - protein, 13 aa, Artificial Sequence
  VH CDR3 of 5H.RA3, 5F.RE6
ARKGARGITGLDY

SEQ ID NO: 75 - protein, 8 aa, Artificial Sequence
  VH CDR1 of 5G.RG1
GFTLSSYG

SEQ ID NO: 76 - protein, 8 aa, Artificial Sequence
  VH CDR2 of 5G.RG1
IWYDGSSK

SEQ ID NO: 77 - protein, 14 aa, Artificial Sequence
  VH CDR3 of 5G.RG1
ARETILIGGVPFDY

SEQ ID NO: 78 - protein, 7 aa, Artificial Sequence
  VL CDR1 of 5G.RG1
QSIRSNY

SEQ ID NO: 79 - protein, 8 aa, Artificial Sequence
  VH CDR1 of 5H.RG4
GYTFTGHY

SEQ ID NO: 80 - protein, 8 aa, Artificial Sequence
  VH CDR2 of 5H.RG4, 5G.RC5
INPNSGGT

SEQ ID NO: 81 - protein, 16 aa, Artificial Sequence
  VH CDR3 of 5H.RG4
ARGYYDTSGYYYAFEF

SEQ ID NO: 82 - protein, 8 aa, Artificial Sequence
  VH CDR1 of 5G.RC5
GYSFIDYY

SEQ ID NO: 83 - protein, 15 aa, Artificial Sequence
  VH CDR3 of 5G.RC5
ARGHCGGDCYCFFDH

SEQ ID NO: 84 - protein, 6 aa, Artificial Sequence
  VL CDR1 of 5F.RE6
QSISNY

SEQ ID NO: 85 - protein, 9 aa, Artificial Sequence
  VL CDR3 of 5F.RE6, 5H.RF2
RQNYNTPLT

SEQ ID NO: 86 - protein, 8 aa, Artificial Sequence
  VH CDR1 of 5H.RF2
GGSLSDYY

SEQ ID NO: 87 - protein, 7 aa, Artificial Sequence
  VH CDR2 of 5H.RF2
INHSGTT

SEQ ID NO: 88 - protein, 16 aa, Artificial Sequence
  VH CDR3 of 5H.RF2
AIEYSNSRGYYYGMDV

SEQ ID NO: 89 - protein, 121 aa, Artificial Sequence
  VH of 5D.RH4
QIQLVESGGGVVQPGRSLRLSCAASGFTFSSDGMHWVRQAPGKGLEWVAVIWFDGRNKYYLDSVKGRFTISRDNSKNTLYLQMNSLRAEDTAVYYCARESSISTRPPFDYWGQGTLVTVSS

SEQ ID NO: 90 - protein, 107 aa, Artificial Sequence
  VL of 5D.RH4
EIVLTQSPGTLSLSPGERATLSCRASQSVRSSYLAWYQQKPGQAPRLLIYGASSRATGIPDRFSGSGSGTDFTLTISRLEPEDFAVYYCQQYGRSYTFGQGTKLEIK

SEQ ID NO: 91 - protein, 123 aa, Artificial Sequence
  VH of 5H.RH4
QVQLQQWGAGLLKPSETLSLTCAVYGGSFSNYYWSWIHQPPGKGLEWIGEINHSGSTNYNPSLKSRVTISVDTSKKQFSLNLSSVTAADTAVYYCKVEHSSSSGHYYYGMDVWGQGTTVTVSS

SEQ ID NO: 92 - protein, 107 aa, Artificial Sequence
  VL of 5H.RH4
DIQMTQSPSSLSASVGDRVTITCRASQTISYYLNWYQQKPGKAPKLLIYAASRLQSGVPSRFSGSGSGTDFTLTISSLQPEDFTTYYCQQSYSTPLTFGGGTKVGIK

SEQ ID NO: 93 - protein, 121 aa, Artificial Sequence
  VH of 5G.RF6
QVQLVESGGGVVQPGRSLRLSCAASGFTFSNYGMHWVRQAPGKGLEWVAVIWYDGSNKYYADSVRGRFTISRDNSKNTQYLQMNSLRAEDTAVYYCARETIMVRGVPFDYWGQGTLVTVSS

SEQ ID NO: 94 - protein, 107 aa, Artificial Sequence
  VL of 5G.RF6
EIVLTQSPGTLSLSPGERATLSCRASQSVRSSYLAWYQQKPGQAPRLLIYGASSRATGIPDRFSGSGSGTDFTLTISRLEPEDFAVYYCQQYGSSYTFGQGTKLEIK

SEQ ID NO: 95 - protein, 121 aa, Artificial Sequence
  VH of 5G.RD6
QVQLVESGGGVVQPGRSLRLSCAASGFAFSSYGMHWVRQAPGKGLEWVAVIWYDGSNRYYADSVKGRFTISRDTSKNTLFLQMNSLRAEDTAVYYCARETAMVRGVPFDYWGQGTLVTVSS

SEQ ID NO: 96 - protein, 107 aa, Artificial Sequence; identical to SEQ ID NO: 94
  VL of 5G.RD6

SEQ ID NO: 97 - protein, 120 aa, Artificial Sequence
  VH of 5H.RA3
QVQLVESGGGVVQPGRSLRVSCAASGFTFSSYGMLWVRQAPGKGLEWVAVIWYDGTKKYYADSLKGRFTISRDNSKYTLYLQMNSLRADDTALYFCARKGARGITGLDYWGQGTLVTVSS

SEQ ID NO: 98 - protein, 107 aa, Artificial Sequence; identical to SEQ ID NO: 94
  VL of 5H.RA3

SEQ ID NO: 99 - protein, 121 aa, Artificial Sequence
  VH of 5G.RG1
QVQLVESGGGVVQPGRSLRLSCVASGFTLSSYGMHWVRQAPGKGLEWVAVIWYDGSSKYYTDSVKGRFDISRDNSKNTLYLQMNILRAEDTAVYYCARETILIGGVPFDYWGQGTLVTVSS

SEQ ID NO: 100 - protein, 107 aa, Artificial Sequence
  VL of 5G.RG1
EIVLTQSPGTLSLSPGERATLSCGASQSIRSNYLAWYQQKPGQAPRLLIYGASSRATGTPDRFSGSGSGTDFTLTITRLEPEDFALYYCQQYGRSYTFGQGTKLEIK

SEQ ID NO: 101 - protein, 123 aa, Artificial Sequence
  VH of 5H.RG4
QVQLVQSGAEVKKPGASVKVSCKASGYTFTGHYFHWVRQAPGQGLEWMGWINPNSGGTNFAQRFQGRVTMTRVTSISTAYMELSGLRSDDTAVYYCARGYYDTSGYYYAFEFWGQGTLVIVSS

SEQ ID NO: 102 - protein, 107 aa, Artificial Sequence; identical to SEQ ID NO: 94
  VL of 5H.RG4

SEQ ID NO: 103 - protein, 122 aa, Artificial Sequence
  VH of 5G.RC5
QVQLVQSGAEVKKPGASVKVSCKASGYSFIDYYMHWVRQAPGQGLEWMGWINPNSGGTNYAQKFQGRVTMTRDTSISTAYMEMRRLRSDDTAVYYCARGHCGGDCYCFFDHWGQGTLVIVSS

SEQ ID NO: 104 - protein, 107 aa, Artificial Sequence
  VL of 5G.RC5
EIVLTQSPGTLSLSPGERATLSCRASQSVRSSYLAWYQQKPGQAPRLLIYDASSRATGTPDRFSGSGSGTDFTLTISRLEPEDFAVYYCQQYGSSYTFGQGTKLEIK

SEQ ID NO: 105 - protein, 120 aa, Artificial Sequence
  VH of 5F.RE6
QVQLAESGGGVVQPGRSLRVSCAASGFTFSSYGMHWVRQAPGKGLEWVAVIWYDGTKKYYADSLKGRFTISRDNSKYTLYLQMNSLRADDTALYFCARKGARGITGLDYWGQGTLVTVSS

SEQ ID NO: 106 - protein, 107 aa, Artificial Sequence
  VL of 5F.RE6
DIQMTQSPSSLSASAGDRITITCRASQSISNYLNWYQQKPGKAPKLLIYAASSLQSGVPSRFSGSGSGTDFTLTISSLQPEDFASYYCRQNYNTPLTFGGGTKVEIK

SEQ ID NO: 107 - protein, 122 aa, Artificial Sequence
  VH of 5H.RF2
QVQLQQWGAGLLKPSETLALTCAVYGGSLSDYYWSWIRQPPGKGLEWIGEINHSGTTNYNPSLKSRVTISVDTSKKQFSLKLSSVTAADTAVYYCAIEYSNSRGYYYGMDVWGQGTTVTVSS

SEQ ID NO: 108 - protein, 107 aa, Artificial Sequence
  VL of 5H.RF2
DIQMTQSPSSLSASAGDRITITCRASQTISNYLNWYQQKPGKAPKLLIYAASSLQSGVPSRFSGSGSGTDFTLTISSLQPEDFASYYCRQNYNTPLTFGGGTKVEIK

SEQ ID NO: 109 - protein, 6 aa, Artificial Sequence
  VL CDR1 of 5H.RF2
QTISNY